European Patent Application EP 4 303 304 A1, published January 10, 2024. Title: Polynucleotides, vectors, cells, pharmaceutical compositions for the treatment of neurodegenerative diseases and a screening method. Applicant: Kyoto Univ. The sequence listing filed with the application follows.

SEQUENCE LISTING (14 sequences)

SEQ ID NO: 1 - DNA, 1491 bp, Homo sapiens
atgaccacatttttcaccagcgtccccccctggattcaagatgcaaagcaggaggaggaagtgggctggaaactagttcccaggcctcggggccgggaggcggagagtcaagtgaagtgccaatgtgaaatttcgggaacacctttctcaaatggggagaagctgaggcctcacagcctcccgcaaccagagcagagaccatatagctgccctcagctgcactgtggcaaggcttttgcttccaaatacaagctgtataggcacatggccacccactcagcccagaaaccccaccagtgtatgtactgtgataagatgtttcaccgcaaggaccatctgcggaaccatctgcagacccatgatcctaacaaagaggccctccactgctctgagtgcggtaagaattacaatacgaagctgggctaccggcgccacctggccatgcatgctgccagcagcggtgacctcagctgcaaggtgtgcctgcagacctttgagagtacccaggccctgctagagcacctgaaggcccactcacgccgggtagcaggcggtgccaaggagaagaagcacccctgtgaccactgcgaccggcggttctatactcgtaaggatgtacggcggcacctagtggtgcacacaggccgtaaggacttcctgtgccagtactgtgcccagcggtttggccgtaaggaccacctgacgcgtcatgtcaagaagagccactcgcaggagctgctcaagatcaagacagagcccgtggacatgttaggcctactcagctgcagctccacagtcagtgtgaaggaagagctgagccctgtgctgtgcatggcctctcgggacgtaatggggaccaaggccttccctggcatgttgcccatgggcatgtatggtgcccacatccctaccatgcccagcacgggcgtgccacactccctggtgcacaacacgctgcccatgggtatgagctaccctctggaatcctcacctatctcttccccagctcagctccctccaaaataccagcttggatctacctcatacttgcccgacaaattgcccaaagtggaggtggatagttttctggcggagcttcctggaagcctgtctctctcatccgctgaaccccagcccgcctcacctcagccggcggcagctgcggccctcctagatgaagcactgcttgccaagagccccgccaacctctctgaggccctctgcgctgctaatgtggacttctcccacctactgggctttcttccactcaacctgcccccgtgtaacccacctggggccacaggaggcctggtcatgggctactcccaggctgaggcacagcccctgcttaccactttgcaagctcagcctcaagattccccaggagctgggggaccactgaactttgggcctctgcactccttgcctcctgtcttcacgtctggcctgagtagcaccaccctgcctcgtttccatcaagcattccagtag

SEQ ID NO: 2 - DNA, 5518 bp, Homo sapiens
gggagcgcggcgcgggagcccgaggctgagactcaccggaggaagcggcgcgagcgccccgccatcgtcccggctgaagtgcagtggcacgatcataggtggtcactacagtctcagattcctgggcttaagcagtcttcccacctcagcctccccagtagctgggattacagtgttatagttttgccgctggactcttccctcccttcccccaccccatcaggatgatatgagacttgaaagaagacgatgcatacaggaggagagacttcagcatgcaaaccttcatctgttcggcttgcaccgtcattttcattccatgctgctggccttcagatggctggacagatgccccattcacatcagtacagtgaccgtcgccagccaaacataagtgaccaacaggtttctgccttatcatattctgaccagattcagcaacctctaactaaccaggtgatgcctgatattgtcatgttacagaggcggatgccccaaaccttccgtgacccagcaactgctcccctgagaaaactttctgttgacttgatcaaaacatacaagcatattaatgaggtttactatgcaaaaaagaagcgaagacaccaacagggccagggagacgattctagtcataagaaggaacggaaggtttacaatgatggttatgatgatgataactatgattatattgtaaaaaacggagaaaagtggatggatcgttacgaaattgactccttgataggcaaaggttcctttggacaggttgtaaaggcatatgatcgtgtggagcaagaatgggttgccattaaaataataaagaacaagaaggcttttctgaatcaagcacagatagaagtgcgacttcttgagctcatgaacaaacatgacactgaaatgaaatactacatagtgcatttgaaacgccactttatgtttcgaaaccatctctgtttagtttttgaaatgctgtcctacaacctctatgacttgctgagaaacaccaatttccgaggggtctctttgaacctaacacgaaagtttgcgcaacagatgtgcactgcactgcttttccttgcgactccagaacttagtatcattcactgtgatctaaaacctgaaaatatccttctttgtaaccccaaacgcagtgcaatcaagatagttgactttggcagttcttgtcagttggggcagaggatataccagtatattcagagtcgcttttatcggtctccagaggtgctactgggaatgccttatgaccttgccattgatatgtggtccctcgggtgtattttggttgaaatgcacactggagaacctctgttcagtggtgccaatgaggtagatcagatgaataaaatagtggaagttctgggtattccacctgctcatattcttgaccaagcaccaaaagcaagaaagttctttgagaagttgccagatggcacttggaacttaaagaagaccaaagatggaaaacgggagtacaaaccaccaggaacccgtaaacttcataacattcttggagtggaaacaggaggacctggtgggcgacgtgctggggagtcaggtcatacggtcgctgactacttgaagttcaaagacctcattttaaggatgcttgattatgaccccaaaactcgaattcaaccttattatgctctgcagcacagtttcttcaagaaaacagctgatgaaggtacaaatacaagtaatagtgtatctacaagccccgccatggagcagtctcagtcttcgggcaccacctccagtacatcgtcaagctcaggtggctcatcggggacaagcaacagtgggagagcccggtcggatccgacgcaccagcatcggcacagtggtgggcacttcacagctgccgtgcaggccatggactgcgagacacacagtccccaggtgagctcgcacgtggttcatttgcttgtgtcacctgccattctcaggtggagcagcactggatgccaggtgcctttagaatgaccgtatcatttaccctagaggttcatgacgttcctgtctaaggaaatgtgcgtcagcaatttcctgctcctcttggttggtcaggcactgaagctcctacacaggtcactgttgaaactcatcctgttcaagaaacaacctttcatgtagcccctcaacagaatgcattgcatcatcaccatggtaacagttcccatcaccatcaccaccaccaccaccatcaccaccaccatggacaacaagccttgggtaaccggaccaggccaagggtctacaattctccaacgaatagctcctctacccaagattctatggaggttggccacagtcaccactccatgacatccctgtcttcctcaacgacttcttcctcgacatcttcctcctctactggtaaccaaggcaatcaggcctaccagaatcgcccagtggctgctaataccttggactttggacagaatggagctatggacgttaatttgaccgtctactccaatccccgccaagagactggcatagctggacatccaacataccaattttctgctaatacaggtcctgcacattacatgactgaaggacatctgacaatgaggcaaggggctgatagagaagagtcccccatgacaggagtttgtgtgcaacagagtcctgtagctagctcgtgactacattgaaacttgagtttgtttcttgtgtgtttttatagaagtggtgttttttttccaaaaacaaagtgcaaagctgcttgaatcaggaggagattaacacactgaaccgctacaagagggcaaagctgattttttttttaacttgaaaagattgcaaagggacattgaagtgtttaaaagagccatgtccaaacccatcttcatggatagctcagaggtatcctctttttgctcccccattttaacttgccacatcccagtcacagtggggtttttttgtctttctattcagcaaaagttaatattcagatgttggtcttggtcatttgccaactaattttaaagtaaaaggcactgcacataatttgcataaagggccccatgagggtgttttttttttttctttttgtcccccccatccccctttttttttgttttgttctgttttgttttgggtgggagggtgggaaatttgggtttttaagtcctctaaacacacttgggcacggaaatgcagtactgtaaggaagagggacctccagcttccacaaacaccatcttcagctgtatgaaagggacggttgtggtgaagtttgtcaggcacagtaagcatgctgagtggcggggatcagaactctcctatctgaacctactgaggagcaaagcagcaattacatgggatcctgtggctctcccgttgcagaggccacaggaagataggatggaacgtgactggtctcctaaccaaggtgcactgagaagcaatcaacgggtcggtcgtggccagtcctggggaggtctgagtggtggtctttgggataacctttggccttatggatttggactcgaaattagaagagcctaccatttcagatgcaatcacttttggacatgcttttgcagacagtccttaatgctgaaaacacagagaatgggtaattcaagaggcctttcttttaaaatagacttttgtgacccactaattgtaaggtattgcaaggtcactttgcgtgtgtcataaagttgacttccttattggttgaaggtcacagaagtagtggtttgctttgatggaaatagctacagctgtgtcccttcctgctttttactttttcttttgctttttctcggcacgtggtatctccaccatttcttctgcacaaagatgtcttctgttcatcctgaacatttttaaaaaatgcagaattttatgtgactgcttttttgcctcacaattatgctgtgaattttacaaaaatttattttcttttttgataatttattgtaccaaagctgtttttatagcacatagatgtctgtaaccaataatgtagcagttctgcactttgacacaaggtgtaactagaccatttttaaatgtcagttgaaaattatggctgtactattgcttaaacaaaactggaactgttgttgaatccatagccaatacatttacagcaatctgtgtactgaacatagtagattgacatctaattcaagattacaacatctgttacattctaagtgtgttcaggcttctgaaggtaaagggacactggatccagaagctatggaaccagcagttgattcttgtattcctgattaacctacttgtaaacttgaaagcaagaccttgattgcaccaacaggtccagagtatgagtgcaagcaaagcagaactctcatgcgtgacctgagcagacaggctggtatttaacaggtgcctcgtgttgagattacgctgccttaatgtaacacagtctggcagttgctaaatttgtgttcccattttaaattgaccaattttggggtgtgacacttttgagcggttgaattgggagaatgaagataagtaatttacctgtccaggatcaaaagaagcctagaaaagaagcagtaatctacctctgccgataacctgtttaagatgactcagcagaacaccgcgtttcattctattggtcaattccatgtggctgactaggtcaattttttttctgaacaaaagcaggtttttatatgtaaacagtgagaaaagaaaggctaaacactatgtaaatgtgaatggaaacttggaaatactcgtttttataaactacaaaaactttttgttgtttatcaggaaatccatatttattttgtaattaactgtcaagcctgtggatgatttttttgaacttggtagttcataaaggtttacagtgaataaaaggatatcatcttgagtatagcaatatcaaaaggaattcagtagttactgctgtttaggaatataaggttaagatatcatatgggtcaggtcattttttttttctgtgctggttgccacatcttagcaagcaccaaaaaactaaagcagtttttaaaccgatatttacgtaaagaaaatcataaaatccaatgcttctgcatactgtgttatgttacagtccagttttgtgtgctttactacacagtttggttacaggacttctgtgcattgtaaacataaacagcatggaaaaggttaaatacctgtgttcagattgtaagatctagtccggacttgctgtgtatattgtaacgttaaatgaaaaaagaacccccctttgtattatagtcatgcggtcttatgtatgataaacagttgaataatttgtcctcagactctttactatgcttttttaaaaattaatttaagaaaaatgtaaacatagtaaaaatcttcctatgcaattaaactggtccaggtctggtaggtatagtatcaaagttgagttaaatgtgtaaaaaggaaactatttgagatacattgacataggcatcagcaatctctgaaagtaaaaattggaggtttaacagat

SEQ ID NO: 3 - DNA, 337 bp, Artificial
  shRNA
tagggataacagggtaattgtttgaatgaggcttcagtactttacagaatcgttgcctgcacatcttggaaacacttgctgggattacttcgacttcttaacccaacagaaggctcgagaaggtatattgctgttgacagtgagcgccctgattaacctacttgtaaatagtgaagccacagatgtatttacaagtaggttaatcaggatgcctactgcctcggacttcaaggggctagaattcgagcaattatcttgtttactaaaactgaataccttgctatctctttgatacatttttacaaagctgaattaaaatggtataaattaaatcact

SEQ ID NO: 4 - DNA, 1506 bp, Homo sapiens
aaggctcctcattggaccctgccagctggccagggaaccccactcctggattcaaactctgcctaaccagccctgatgccagccccagctctgggggctaaggcccttccgctaggacccggcagggtcccaacctgtctctaggagccagcccaggccccgaatcctctcctagtctctgctgcagagcatttgaggaactgtgaccgcaggctagggggtgggggtctcccaagggaccctcccctaaggacccagggtgggattcattgcctcaaagtggctgcgggcactcagctcagttggccaggtaccggggttattagctcatcccatggaccggtggttgggggcggggggctagggctggcatggcctctgatcctcaagtctgccacctggcacccactccctacccactggcaaaatgccagaggaaagcaagccctacaagtgccctggctgccagagagactaggtggagctgtggcatgcataaacagtggccacagcaagcatgccaagagccgaggcctcccgagctgcgtggacactgtagtcagatccctggccagataggggtggggagaggcccctgagggacacctgccagctcgtggagcagccccagtgctgctgtgggttacagtgctcctgggaggacagggtgcaggaagcggggagagctgccgggtgcccggctccgcggggagagctgccgggtgccgggctccacgtggagcacgggccccagcttcctggagctgcccggagcccagccaggaaggcacaaggcccattttctaggtctggagaagtcaggagtcccaggtgacagtcagggggcttgtaatataggcacgtaggactgatcctaagagcgtcgccccctctgtccccctcccctggaggggcagcaggtcccagtcagggaaggtgcccatcccccaggaagccgtggcacttgttcattctacagtttttcccttatctgctcctacggcctctgccagccagcagtgggaagccgctggggagaggcaggggaggggagcggaggggagggcgggggagggggccctccttcctgcccccctcccgtttggcggcctgggaaaaggcagcatattgaggcgcggggctcccggcatcaggccccgggatgctaatgagggcgagcgcgttcccacagcccggacattgtgccgcgcggcccacctgctccttggggagcgcccattgtgcccgcgccaattcacaggcaatttagcgtgcgctaatgggccggcgcctttgtgcggcccgcccggccattggccgcggagtgtgggaacggccgcggcgcccggactccaggcgccaggccgccgcccgcgcctatatagggcgtcggcgcgcggggccggtgtccgcgccagcccgggacgcgcttggccttgcccgcgcccgctcgcctcgtctcgcccggcctccccgcgtcgcctcgtcgcctgttccgcgccaggc

SEQ ID NO: 5 - DNA, 4227 bp, Homo sapiens
aaggctcctcattggaccctgccagctggccagggaaccccactcctggattcaaactctgcctaaccagccctgatgccagccccagctctgggggctaaggcccttccgctaggacccggcagggtcccaacctgtctctaggagccagcccaggccccgaatcctctcctagtctctgctgcagagcatttgaggaactgtgaccgcaggctagggggtgggggtctcccaagggaccctcccctaaggacccagggtgggattcattgcctcaaagtggctgcgggcactcagctcagttggccaggtaccggggttattagctcatcccatggaccggtggttgggggcggggggctagggctggcatggcctctgatcctcaagtctgccacctggcacccactccctacccactggcaaaatgccagaggaaagcaagccctacaagtgccctggctgccagagagactaggtggagctgtggcatgcataaacagtggccacagcaagcatgccaagagccgaggcctcccgagctgcgtggacactgtagtcagatccctggccagataggggtggggagaggcccctgagggacacctgccagctcgtggagcagccccagtgctgctgtgggttacagtgctcctgggaggacagggtgcaggaagcggggagagctgccgggtgcccggctccgcggggagagctgccgggtgccgggctccacgtggagcacgggccccagcttcctggagctgcccggagcccagccaggaaggcacaaggcccattttctaggtctggagaagtcaggagtcccaggtgacagtcagggggcttgtaatataggcacgtaggactgatcctaagagcgtcgccccctctgtccccctcccctggaggggcagcaggtcccagtcagggaaggtgcccatcccccaggaagccgtggcacttgttcattctacagtttttcccttatctgctcctacggcctctgccagccagcagtgggaagccgctggggagaggcaggggaggggagcggaggggagggcgggggagggggccctccttcctgcccccctcccgtttggcggcctgggaaaaggcagcatattgaggcgcggggctcccggcatcaggccccgggatgctaatgagggcgagcgcgttcccacagcccggacattgtgccgcgcggcccacctgctccttggggagcgcccattgtgcccgcgccaattcacaggcaatttagcgtgcgctaatgggccggcgcctttgtgcggcccgcccggccattggccgcggagtgtgggaacggccgcggcgcccggactccaggcgccaggccgccgcccgcgcctatatagggcgtcggcgcgcggggccggtgtccgcgccagcccgggacgcgcttggccttgcccgcgcccgctcgcctcgtctcgcccggcctccccgcgtcgcctcgtcgcctgttccgcgccaggcttaattaagccaccatgaccacatttttcaccagcgtccccccctggattcaagatgcaaagcaggaggaggaagtgggctggaaactagttcccaggcctcggggccgggaggcggagagtcaagtgaagtgccaatgtgaaatttcgggaacacctttctcaaatggggagaagctgaggcctcacagcctcccgcaaccagagcagagaccatatagctgccctcagctgcactgtggcaaggcttttgcttccaaatacaagctgtataggcacatggccacccactcagcccagaaaccccaccagtgtatgtactgtgataagatgtttcaccgcaaggaccatctgcggaaccatctgcagacccatgatcctaacaaagaggccctccactgctctgagtgcggtaagaattacaatacgaagctgggctaccggcgccacctggccatgcatgctgccagcagcggtgacctcagctgcaaggtgtgcctgcagacctttgagagtacccaggccctgctagagcacctgaaggcccactcacgccgggtagcaggcggtgccaaggagaagaagcacccctgtgaccactgcgaccggcggttctatactcgtaaggatgtacggcggcacctagtggtgcacacaggccgtaaggacttcctgtgccagtactgtgcccagcggtttggccgtaaggaccacctgacgcgtcatgtcaagaagagccactcgcaggagctgctcaagatcaagacagagcccgtggacatgttaggcctactcagctgcagctccacagtcagtgtgaaggaagagctgagccctgtgctgtgcatggcctctcgggacgtaatggggaccaaggccttccctggcatgttgcccatgggcatgtatggtgcccacatccctaccatgcccagcacgggcgtgccacactccctggtgcacaacacgctgcccatgggtatgagctaccctctggaatcctcacctatctcttccccagctcagctccctccaaaataccagcttggatctacctcatacttgcccgacaaattgcccaaagtggaggtggatagttttctggcggagcttcctggaagcctgtctctctcatccgctgaaccccagcccgcctcacctcagccggcggcagctgcggccctcctagatgaagcactgcttgccaagagccccgccaacctctctgaggccctctgcgctgctaatgtggacttctcccacctactgggctttcttccactcaacctgcccccgtgtaacccacctggggccacaggaggcctggtcatgggctactcccaggctgaggcacagcccctgcttaccactttgcaagctcagcctcaagattccccaggagctgggggaccactgaactttgggcctctgcactccttgcctcctgtcttcacgtctggcctgagtagcaccaccctgcctcgtttccatcaagcattccagggaagcggagctactaacttcagcctgctgaagcaggctggagacgtggaggagaaccctggacctgtgagcaagggcgaggaggataacatggccatcatcaaggagttcatgcgcttcaaggtgcacatggagggctccgtgaacggccacgagttcgagatcgagggcgagggcgagggccgcccctacgagggcacccagaccgccaagctgaaggtgaccaagggtggccccctgcccttcgcctgggacatcctgtcccctcagttcatgtacggctccaaggcctacgtgaagcaccccgctgacatccccgactacttgaagctgtccttccccgagggcttcaagtgggagcgcgtgatgaacttcgaggacggcggcgtggtgaccgtgacccaggactcctccctgcaggacggcgagttcatctacaaggtgaagctgcgcggcaccaacttcccctccgacggccccgtaatgcagaagaagaccatgggctgggaggcctcctccgagcggatgtaccccgaggacggcgccctgaagggcgagatcaagcagaggctgaagctgaaggacggcggccactacgacgctgaggtcaagaccacctacaaggccaagaagcccgtgcagctgcccggcgcctacaacgtcaacatcaagttggacatcacctcccacaacgaggactacaccatcgtggaacagtacgaacgcgccgagggccgccactccaccggcggcatggacgagctgtacaaggatatccctccaaagaagaagagaaaggtgtaaggcgcgcctagggataacagggtaattgtttgaatgaggcttcagtactttacagaatcgttgcctgcacatcttggaaacacttgctgggattacttcgacttcttaacccaacagaaggctcgagaaggtatattgctgttgacagtgagcgccctgattaacctacttgtaaatagtgaagccacagatgtatttacaagtaggttaatcaggatgcctactgcctcggacttcaaggggctagaattcgagcaattatcttgtttactaaaactgaataccttgctatctctttgatacatttttacaaagctgaattaaaatggtataaattaaatcactctagtaataaaggatcctttatcttcattggatccgtgtgttggttttttgtgtgcggcccgtctagacc

SEQ ID NO: 6 - DNA, 3011 bp, Homo sapiens
aaggctcctcattggaccctgccagctggccagggaaccccactcctggattcaaactctgcctaaccagccctgatgccagccccagctctgggggctaaggcccttccgctaggacccggcagggtcccaacctgtctctaggagccagcccaggccccgaatcctctcctagtctctgctgcagagcatttgaggaactgtgaccgcaggctagggggtgggggtctcccaagggaccctcccctaaggacccagggtgggattcattgcctcaaagtggctgcgggcactcagctcagttggccaggtaccggggttattagctcatcccatggaccggtggttgggggcggggggctagggctggcatggcctctgatcctcaagtctgccacctggcacccactccctacccactggcaaaatgccagaggaaagcaagccctacaagtgccctggctgccagagagactaggtggagctgtggcatgcataaacagtggccacagcaagcatgccaagagccgaggcctcccgagctgcgtggacactgtagtcagatccctggccagataggggtggggagaggcccctgagggacacctgccagctcgtggagcagccccagtgctgctgtgggttacagtgctcctgggaggacagggtgcaggaagcggggagagctgccgggtgcccggctccgcggggagagctgccgggtgccgggctccacgtggagcacgggccccagcttcctggagctgcccggagcccagccaggaaggcacaaggcccattttctaggtctggagaagtcaggagtcccaggtgacagtcagggggcttgtaatataggcacgtaggactgatcctaagagcgtcgccccctctgtccccctcccctggaggggcagcaggtcccagtcagggaaggtgcccatcccccaggaagccgtggcacttgttcattctacagtttttcccttatctgctcctacggcctctgccagccagcagtgggaagccgctggggagaggcaggggaggggagcggaggggagggcgggggagggggccctccttcctgcccccctcccgtttggcggcctgggaaaaggcagcatattgaggcgcggggctcccggcatcaggccccgggatgctaatgagggcgagcgcgttcccacagcccggacattgtgccgcgcggcccacctgctccttggggagcgcccattgtgcccgcgccaattcacaggcaatttagcgtgcgctaatgggccggcgcctttgtgcggcccgcccggccattggccgcggagtgtgggaacggccgcggcgcccggactccaggcgccaggccgccgcccgcgcctatatagggcgtcggcgcgcggggccggtgtccgcgccagcccgggacgcgcttggccttgcccgcgcccgctcgcctcgtctcgcccggcctccccgcgtcgcctcgtcgcctgttccgcgccaggcttaattaagccaccatgaccacatttttcaccagcgtccccccctggattcaagatgcaaagcaggaggaggaagtgggctggaaactagttcccaggcctcggggccgggaggcggagagtcaagtgaagtgccaatgtgaaatttcgggaacacctttctcaaatggggagaagctgaggcctcacagcctcccgcaaccagagcagagaccatatagctgccctcagctgcactgtggcaaggcttttgcttccaaatacaagctgtataggcacatggccacccactcagcccagaaaccccaccagtgtatgtactgtgataagatgtttcaccgcaaggaccatctgcggaaccatctgcagacccatgatcctaacaaagaggccctccactgctctgagtgcggtaagaattacaatacgaagctgggctaccggcgccacctggccatgcatgctgccagcagcggtgacctcagctgcaaggtgtgcctgcagacctttgagagtacccaggccctgctagagcacctgaaggcccactcacgccgggtagcaggcggtgccaaggagaagaagcacccctgtgaccactgcgaccggcggttctatactcgtaaggatgtacggcggcacctagtggtgcacacaggccgtaaggacttcctgtgccagtactgtgcccagcggtttggccgtaaggaccacctgacgcgtcatgtcaagaagagccactcgcaggagctgctcaagatcaagacagagcccgtggacatgttaggcctactcagctgcagctccacagtcagtgtgaaggaagagctgagccctgtgctgtgcatggcctctcgggacgtaatggggaccaaggccttccctggcatgttgcccatgggcatgtatggtgcccacatccctaccatgcccagcacgggcgtgccacactccctggtgcacaacacgctgcccatgggtatgagctaccctctggaatcctcacctatctcttccccagctcagctccctccaaaataccagcttggatctacctcatacttgcccgacaaattgcccaaagtggaggtggatagttttctggcggagcttcctggaagcctgtctctctcatccgctgaaccccagcccgcctcacctcagccggcggcagctgcggccctcctagatgaagcactgcttgccaagagccccgccaacctctctgaggccctctgcgctgctaatgtggacttctcccacctactgggctttcttccactcaacctgcccccgtgtaacccacctggggccacaggaggcctggtcatgggctactcccaggctgaggcacagcccctgcttaccactttgcaagctcagcctcaagattccccaggagctgggggaccactgaactttgggcctctgcactccttgcctcctgtcttcacgtctggcctgagtagcaccaccctgcctcgtttccatcaagcattccagtag

SEQ ID NO: 7 - DNA, 1921 bp, Artificial Sequence
  promotor_shRNA
aaggctcctcattggaccctgccagctggccagggaaccccactcctggattcaaactctgcctaaccagccctgatgccagccccagctctgggggctaaggcccttccgctaggacccggcagggtcccaacctgtctctaggagccagcccaggccccgaatcctctcctagtctctgctgcagagcatttgaggaactgtgaccgcaggctagggggtgggggtctcccaagggaccctcccctaaggacccagggtgggattcattgcctcaaagtggctgcgggcactcagctcagttggccaggtaccggggttattagctcatcccatggaccggtggttgggggcggggggctagggctggcatggcctctgatcctcaagtctgccacctggcacccactccctacccactggcaaaatgccagaggaaagcaagccctacaagtgccctggctgccagagagactaggtggagctgtggcatgcataaacagtggccacagcaagcatgccaagagccgaggcctcccgagctgcgtggacactgtagtcagatccctggccagataggggtggggagaggcccctgagggacacctgccagctcgtggagcagccccagtgctgctgtgggttacagtgctcctgggaggacagggtgcaggaagcggggagagctgccgggtgcccggctccgcggggagagctgccgggtgccgggctccacgtggagcacgggccccagcttcctggagctgcccggagcccagccaggaaggcacaaggcccattttctaggtctggagaagtcaggagtcccaggtgacagtcagggggcttgtaatataggcacgtaggactgatcctaagagcgtcgccccctctgtccccctcccctggaggggcagcaggtcccagtcagggaaggtgcccatcccccaggaagccgtggcacttgttcattctacagtttttcccttatctgctcctacggcctctgccagccagcagtgggaagccgctggggagaggcaggggaggggagcggaggggagggcgggggagggggccctccttcctgcccccctcccgtttggcggcctgggaaaaggcagcatattgaggcgcggggctcccggcatcaggccccgggatgctaatgagggcgagcgcgttcccacagcccggacattgtgccgcgcggcccacctgctccttggggagcgcccattgtgcccgcgccaattcacaggcaatttagcgtgcgctaatgggccggcgcctttgtgcggcccgcccggccattggccgcggagtgtgggaacggccgcggcgcccggactccaggcgccaggccgccgcccgcgcctatatagggcgtcggcgcgcggggccggtgtccgcgccagcccgggacgcgcttggccttgcccgcgcccgctcgcctcgtctcgcccggcctccccgcgtcgcctcgtcgcctgttccgcgccaggcttaattaatagggataacagggtaattgtttgaatgaggcttcagtactttacagaatcgttgcctgcacatcttggaaacacttgctgggattacttcgacttcttaacccaacagaaggctcgagaaggtatattgctgttgacagtgagcgccctgattaacctacttgtaaatagtgaagccacagatgtatttacaagtaggttaatcaggatgcctactgcctcggacttcaaggggctagaattcgagcaattatcttgtttactaaaactgaataccttgctatctctttgatacatttttacaaagctgaattaaaatggtataaattaaatcactctagtaataaaggatcctttatcttcattggatccgtgtgttggttttttgtgtgcggcccgtctagacc

SEQ ID NO: 8 - DNA, 21 bp, Artificial Sequence
  SiRNA
cctgattaacctacttgtaaa

SEQ ID NO: 9 - DNA, 1618 bp, Mus musculus
tgcacttatatcttgcactggacagaccatcctgtgctgcctcaaagccaagccttcccctctgtcccagatgcttccatccatggtaacccaacaaccccttgtgctaagagcttctggagcaagaccttcggaatagatcatttacagcagtgggtcactaccatagcaggagggcgtttccctagtgggcactgtgaaggcccttcagttcctgagctcagacatggctgacatccatccagagaacctggtttcattccacactggctattgtgctctgatgccagcctcctggtttgggcctggctaggtcttaggttgaccctaggaggaagcacggggccttatctcctccctcagcccctgcagagtattggggaaatagtacaggttccagatggagggacgctcctacatggccatcccctaggtgtctagggtgtgactagtaaggtcacctggttaggaaccacggttatcagttcttacaaagaggcccatccacactggcacagcattcatatgggggcttatttttaggtctcccaccttctacctgccaacacaaaatgctgaatgaaactggaacacacacacagaggcatgcacgcgcgcgcccgcacgagctgagggggatgtcatgagaggagttaagggcagccatggtttcctaaaagccacgcgggagtagtgatcacggacagcatgaaggaggcacggtcctcctgtttcagagatgcatgtggcacctggtgacacaagagcagtccagataccctgtgggttcaggggttcctgagggcttcctaggtatggggctttgtgctaggcattatccaaagcaaattcagctagcctagaagtacgcttggcaggctccgcgcgtggccatttctagctgcggagaagtcactcctctcaactgacagaactggcaataaagcgcctaaattctaaatacatgagtccctctctcatcctgtacctgcgaatggcatggcggcagcatctgtttgagagaatgtggcccactttaacccactgtgcctgtgggcaacaggtcccagctggggagggtgcccactcctctggaagtcgctgtctgttcattgtaaaactctcatttctctgcgcctgtggcctctgccagccagcggtggggagcctctggggagtgggagggaagaagggagagaagggggggggagagcactccttcctgccctccccacctccccgcggcctgggaaaaggcagcatattgaggcgcggggctctcagcatcaggccccgggatgctaatgagggcgagcgcgttcccacagcccggacattgtgccgcgcggcccacctgctcctcggggagcgaccattgtgcccgcgccaattcacaggcaatttagcgtgcgctaatgggccggcgcctttgtgcggccggcgccgccattggccgccgagtgtgggaacggccgcggcgcccggaccccaggcgccgggccgctgcccgcgcctatatagggctggcgtgctggggtccaggtcgcgccagtccgggacgcctggctctgtccgctccgctccgctccgctcgctaatcgcctccagagctccaggc

SEQ ID NO: 10 - DNA, 1491 bp, Mus musculus
atgaccacatttttcaccagcgtccctccctggattcaagatgcaaagcaggaggaggaagtgggctggaaactagttcccaggcctcggggccgggaggcagagagtcaagtgaagtgccaatgtgaaatctcggggacaccattttcaaatggggagaagctaaggcctcacagccttccccatccggagcagagaccatatagctgtcctcagctgcactgcggcaaggcttttgcctccaagtacaagctgtataggcacatggccacccactcggcccagaaaccccaccagtgcatgtactgtgacaagatgtttcaccgaaaggaccatctgcggaaccacttgcagacccatgaccccaacaaagaggccctccactgctctgagtgtggtaagaattataatacaaagctgggataccgtcgtcacctggccatgcatgctgccagcagtggtgatctcagctgcaaggtgtgcctgcagacctttgagagtacccaggccctattggagcacctgaaggctcactcacgccgggtagcaggaggtgctaaggagaagaagcacccctgtgaccattgtgacaggcggttctatactcggaaggatgtccgacggcacctagtggtgcacacaggtcgtaaggacttcctgtgtcagtactgtgcccagagatttggccgcaaggatcacctgacacgccatgtcaagaagagccactcacaggaactgctcaagatcaagacagagccagtggatatgttaggcttgctcagctgtagctctacagtcagtgtaaaggaagagctgagccctgtgctttgcatggcctctcgggacgtgatgggggctaaggcctttcctggcatgttgcccatgggtatgtatggtgcccacatccctaccatgcccagtgcgggcatgccacactccctggtgcacaacacactgcccatgggtatgagttaccctctggaatcttctcctatctcctcctcagctcagctccctccaaaataccagcttggatctacctcatacttgcccgacaaactgcccaaagtggaggtggatagttttctggcagagcttcctggaagcctgtctctctcctcggctgaacctcagcccgcctcacctcagccggcggcagctgcagccctcctggatgaagcactgctcgccaagagtcccgccaacctctccgaggccctctgcgctgctaatgtggacttttcccacttactgggctttcttccgctcaacctacccccatgtaacccaccaggggccacaggaggcttggttatgggctactcccaagctgaggcacagcctttgctcaccactttgcaggctcagcctcaagattccgctggagctgggggacccctgaactttgggcctctgcactccttacctcctgtcttcacctctggcctgagtaccaccaccctgcctcgtttccaccaagcattccagtag

SEQ ID NO: 11 - DNA, 3141 bp, Mus musculus
tgcacttatatcttgcactggacagaccatcctgtgctgcctcaaagccaagccttcccctctgtcccagatgcttccatccatggtaacccaacaaccccttgtgctaagagcttctggagcaagaccttcggaatagatcatttacagcagtgggtcactaccatagcaggagggcgtttccctagtgggcactgtgaaggcccttcagttcctgagctcagacatggctgacatccatccagagaacctggtttcattccacactggctattgtgctctgatgccagcctcctggtttgggcctggctaggtcttaggttgaccctaggaggaagcacggggccttatctcctccctcagcccctgcagagtattggggaaatagtacaggttccagatggagggacgctcctacatggccatcccctaggtgtctagggtgtgactagtaaggtcacctggttaggaaccacggttatcagttcttacaaagaggcccatccacactggcacagcattcatatgggggcttatttttaggtctcccaccttctacctgccaacacaaaatgctgaatgaaactggaacacacacacagaggcatgcacgcgcgcgcccgcacgagctgagggggatgtcatgagaggagttaagggcagccatggtttcctaaaagccacgcgggagtagtgatcacggacagcatgaaggaggcacggtcctcctgtttcagagatgcatgtggcacctggtgacacaagagcagtccagataccctgtgggttcaggggttcctgagggcttcctaggtatggggctttgtgctaggcattatccaaagcaaattcagctagcctagaagtacgcttggcaggctccgcgcgtggccatttctagctgcggagaagtcactcctctcaactgacagaactggcaataaagcgcctaaattctaaatacatgagtccctctctcatcctgtacctgcgaatggcatggcggcagcatctgtttgagagaatgtggcccactttaacccactgtgcctgtgggcaacaggtcccagctggggagggtgcccactcctctggaagtcgctgtctgttcattgtaaaactctcatttctctgcgcctgtggcctctgccagccagcggtggggagcctctggggagtgggagggaagaagggagagaagggggggggagagcactccttcctgccctccccacctccccgcggcctgggaaaaggcagcatattgaggcgcggggctctcagcatcaggccccgggatgctaatgagggcgagcgcgttcccacagcccggacattgtgccgcgcggcccacctgctcctcggggagcgaccattgtgcccgcgccaattcacaggcaatttagcgtgcgctaatgggccggcgcctttgtgcggccggcgccgccattggccgccgagtgtgggaacggccgcggcgcccggaccccaggcgccgggccgctgcccgcgcctatatagggctggcgtgctggggtccaggtcgcgccagtccgggacgcctggctctgtccgctccgctccgctccgctcgctaatcgcctccagagctccaggccttaagaggcaggcaggcttaattaagccaccatgaccacatttttcaccagcgtccctccctggattcaagatgcaaagcaggaggaggaagtgggctggaaactagttcccaggcctcggggccgggaggcagagagtcaagtgaagtgccaatgtgaaatctcggggacaccattttcaaatggggagaagctaaggcctcacagccttccccatccggagcagagaccatatagctgtcctcagctgcactgcggcaaggcttttgcctccaagtacaagctgtataggcacatggccacccactcggcccagaaaccccaccagtgcatgtactgtgacaagatgtttcaccgaaaggaccatctgcggaaccacttgcagacccatgaccccaacaaagaggccctccactgctctgagtgtggtaagaattataatacaaagctgggataccgtcgtcacctggccatgcatgctgccagcagtggtgatctcagctgcaaggtgtgcctgcagacctttgagagtacccaggccctattggagcacctgaaggctcactcacgccgggtagcaggaggtgctaaggagaagaagcacccctgtgaccattgtgacaggcggttctatactcggaaggatgtccgacggcacctagtggtgcacacaggtcgtaaggacttcctgtgtcagtactgtgcccagagatttggccgcaaggatcacctgacacgccatgtcaagaagagccactcacaggaactgctcaagatcaagacagagccagtggatatgttaggcttgctcagctgtagctctacagtcagtgtaaaggaagagctgagccctgtgctttgcatggcctctcgggacgtgatgggggctaaggcctttcctggcatgttgcccatgggtatgtatggtgcccacatccctaccatgcccagtgcgggcatgccacactccctggtgcacaacacactgcccatgggtatgagttaccctctggaatcttctcctatctcctcctcagctcagctccctccaaaataccagcttggatctacctcatacttgcccgacaaactgcccaaagtggaggtggatagttttctggcagagcttcctggaagcctgtctctctcctcggctgaacctcagcccgcctcacctcagccggcggcagctgcagccctcctggatgaagcactgctcgccaagagtcccgccaacctctccgaggccctctgcgctgctaatgtggacttttcccacttactgggctttcttccgctcaacctacccccatgtaacccaccaggggccacaggaggcttggttatgggctactcccaagctgaggcacagcctttgctcaccactttgcaggctcagcctcaagattccgctggagctgggggacccctgaactttgggcctctgcactccttacctcctgtcttcacctctggcctgagtaccaccaccctgcctcgtttccaccaagcattccagtag

SEQ ID NO: 12 - DNA, 5759 bp, Mus musculus
gcgagggcgagtgtgcgcgcggtgagtgtgcgcgagtgtctgtgcgggatcgggggcgggcggtccgggctctcctggcggagccgccgccgccgccgccgccgctcgggccccggcgctgctcgctgcgcagcttcggagcgcgcgccattttgtgagatttacaaaaatcctcgtcgggaagaagcggccggcagcggccgccactcggcgcccggcctcgccgccgccgccgccctccgcaccgggccgggccgggccccgccgccgacactcgggggcccggggactgcggtatttgccggggaggggctgtcgcctgcctccccggccgcgggcgccgccggccccgccagcccgacggaccctgagccagcgcggctgcggcgcggagccgggacgccgggggcggagagaggcggccggggcggcgctggctgcggaggccgcggcgggagcgcggcgcgggagctcgaggctgagactcaccggagggagcggcgcgagcgccccgccatcgtcccgtgttatagttttgccgctggactcttccctcccttcccccaccccatcaggatgatatgagacttgaaagaagacgatgcatacaggaggagagacttcagcatgcaaaccttcatctgtccggcttgcaccgtcgttctcattccatgctgctggccttcagatggctgcacagatgccccactcacaccagtacagtgaccgtcgccagccgagcataagtgaccagcaggtgtctgccttaccatattctgaccagattcagcaacctctaactaaccaggtgatgcctgacattgtcatgttacagaggcggatgccccaaaccttccgtgatccagcaactgctcctctgagaaaactctctgtggacttgatcaaaacatacaagcatattaatgaggtttactatgcaaaaaagaagcgaagacaccaacagggccagggggacgattccagtcataagaaggagcggaaggtttacaatgatggttacgatgatgataactatgattatattgtaaaaaacggggaaaagtggatggatcggtatgaaatcgactccttaataggcaaaggttcatttggacaggttgtgaaagcttatgacagagtggagcaagaatgggtcgccattaaaatcatcaagaacaagaaagcgtttctgaatcaagcccagatagaagtgcggctgcttgagctcatgaacaaacacgacactgaaatgaagtactacatagtgcatttgaaacgccactttatgtttcgaaaccatctctgtttagtgtttgaaatgctgtcctataatctctatgatttgttgagaaacaccaacttccgaggggtctctttgaacctaacacgaaagtttgcgcaacagatgtgcacagcattgctttttcttgcgactccagaacttagtatcattcactgtgacttaaagcctgagaacatccttctgtgtaaccccaaacggagtgcaatcaagattgttgattttggcagctcttgtcagttggggcagaggatataccagtatattcagagtcgcttttatcggtctccagaggtgctactgggaatgccttatgaccttgctatcgacatgtggtcccttggatgtatcttggttgaaatgcacactggagagcctctgttcagtggtgccaatgaggtcgatcagatgaataaaatagtggaagtcttgggcatcccacctgctcatattcttgaccaagcaccgaaagcaagaaagttctttgagaagttgcccgatggcacttggagcttaaagaagaccaaagatggaaaacgggagtacaaaccaccaggaacccgtaaacttcataatattcttggagtagaaacaggaggacctggcgggcggcgtgctggggaatcgggtcatactgtagctgactacttgaagttcaaagacctcattttaaggatgcttgattatgaccccaaaactcggattcaaccttattatgccctgcagcacagttttttcaagaaaacagctgatgaaggtaccaacacaagtaacagtgtgtctaccagccctgcgatggagcagtctcagtcttcaggcaccacctccagcacctcctccagctcaggtggatcctcgggaacgagtaacagtgggagagccaggtcggatccgacgcaccagcatcgacacagcggtggacacttcgctgctgctgtccaggccatggactgtgagacacacagtccccaggtgcgccagcagtttccggctcctctgggatggtcaggcactgaagctcctacacaagtcactgttgaaactcatcctgttcaagagacaacctttcatgtagccccccagcagaacgcattgcatcatcaccatggaaacagttcccatcaccaccaccaccaccatcaccaccaccaccaccatggacagcaagccttgggtaaccggaccaggccaagggtctacaattctccaacaaatagctcctctacccaggattctatggaggttggccacagtcaccactccatgacatccctgtcttcctcaacaacttcttcctcgacatcttcctcctctactggtaatcaaggcaatcaggcctatcagaaccgcccagtggctgctaacaccttggactttggacagaatggagctatggacgttaatttgaccgtctactccaatccccgccaagagactggcatagctggacatccaacataccaattttctgctaatacaggtcctgcacattacatgactgaaggacatctggcgatgagacaaggggctgatagagaagagtctcccatgacaggagtttgtgtgcaacagagtcctgtagctagctcgtgactacattgaaacttgagtttgtttcttgtgtgtttttatagaagtggtgtttttttcccaaaaaacaaaagtgcaaagctgcttgaatcagaaggagattaacacactgaaccgctacaagagggcaaagctgacttttttttttaacttgaaaagattgcaaagggacaatgaagtttttaagagccatgtccacccatcttcacggagagctcagagtgtcctctttctgcctcccccatttaacttccatctcctggtcacagtgggttttgtctttctatccaacaagagttaatgttcagctgttggtcttggtcatttgccaactaattttaaaataaaaaggcactgcacataatttgcataaagggccccataagggtgttttgttttgttttcatttttattttttccctttttcccttgttttgttttgtttcattttgggctgggggtggggtgggaaatttgggttttttatgtcctctacacacttgggcacggaaatgcagtactgtaaggaagagggacctctagcacacacaaacatcatcttcagctgtgtgaaagggacgattgtgttgacatttgtaaggcacattaagcatgctaagtggcggggatcaggactctcctatctgagcctactgaggagcaaagcagccattgcatgggatcctgtgggtctcctgctggagaggccacaggaggataggatggaacgtgactggtcggtctccttaccaaggcgcactgagaagcaatcagcgggtcggttgtggccagtcctggggaggtctgagtggtggtccttgggataacctttggccttacggatttggactcggagttagaagagcccaccatttcagatgcaatcacttgtggacatgcgtttgcagacagtccttaatgctgaaaacacagagaatgggtaattcaagaggcctttcttttaaaatagacttttgtgacccactaattgtaaggtattgcaaggtcactttgcgtgtgtcataaagctgactcccttcttggttgaaggccacagaggtagtggtttgctttgatggaaatagctacagctgtgtcccttcctgcttttcccttttctttggctttttctcggcacgtggtgtctccaccatttcttctgcacaaagacgtcttctgttcaccctgaacattttaaaatgcagaattttatgtgactgcttttttgcctcacaattatgctgtgaattttacaaaaatttattttcttttttgataatttattgtaccaaagctgtttttatagcacatagatgtctgtaaccaataatgtcgcaggcctgcactttgacacaggtgtaacgagaccgttttaaacgtcagttgaaatgatggctgtactattgcttaaacaaaactggaactgttgttgaatccatagccaatacatttacagcaatcttgtactggacagaatagattgacatctaattcaagattacaacacctgtcacattctaaatgtgttcaggcttctgaagggaaagggacactggatccagaagctatggagccagcagttgatcttgtattcctgattaacttccttgtaaacttgaacttgagaccttgattgaaccgacaggtccacagtaggaacaggaagcaggcagagctctgagcatgacctgaaggaagcaggctggcactagcagttgccttgtctggagatgctgctgccttcaagtagcacagtctggcagtggctaaatctgtgttcccattgaaattgagcaattttagggtgttatactctgaagcagttgaattgggagaatgaagatagagtaatttccctgtccaggatcaaaagaagcctagaaagaagcagtgatctacctctgccaataaccctgttggaagcaacgcagcagaacaccacggtactttttattgcttaattccacgtggctgactaggtcaaggtttgtttggtgttttttttttttttttttgtttctgagcaaaagcaggtttttttttgttttttatatgtaaacaaaagaaaggcctaagctctgtgagtgcaagtggagactcagagagccccgtttctataaacacagacacttcaggtgttaatcaggaaacccatattgattttgtaattaaatgtcaagcctgtggattgttttgagcttggtagttgatgagcatttccgtacagaggcctcaccttgagcacagcactgtcaggagggcgcagcgcctgtggctgcggagccccaggtgccacacacccaccccacgtggctcaggtcattctttttttctttctgtgctggttgccacattttagcaagcaccaaaaaagaaagcagtttttaaagctatatttacgtaaagagagccacacaatccagtgcttctgcataccgtgtcacgttacagtccagttttgtgtgctttactacacagtttggttacaggacttctgtgcattgtaaacataaacagcatggagaggttaaatacctgtgttcagattgtaagatctagtccagacttgctgtgtatattgtaacgttaaatgaaaaaagacccccctttgtattatagtcatgcggtcttatgtatgataaacagttgaataatttgtcctcagagtctttactatgcttttttaaaaattaacttaaggaaaaatgtaaacagtaaaaaaacaatcttcgtgtgcagtgaagcgggtccgggtgtggtaggtaaagcaggcacaatcctgtcgcctatgtaaagggaaaagacttgtgagacagagacattggctgcaagtgtctttgaaagtaaaaattggaggtttaacagataa

SEQ ID NO: 13 - DNA, 337 bp, Artificial Sequence
  shRNA
tagggataacagggtaattgtttgaatgaggcttcagtactttacagaatcgttgcctgcacatcttggaaacacttgctgggattacttcgacttcttaacccaacagaaggctcgagaaggtatattgctgttgacagtgagcgcgctgtgtatattgtaacgttatagtgaagccacagatgtataacgttacaatatacacagcatgcctactgcctcggacttcaaggggctagaattcgagcaattatcttgtttactaaaactgaataccttgctatctctttgatacatttttacaaagctgaattaaaatggtataaattaaatcact

SEQ ID NO: 14 - DNA, 4357 bp, Mus musculus
tgcacttatatcttgcactggacagaccatcctgtgctgcctcaaagccaagccttcccctctgtcccagatgcttccatccatggtaacccaacaaccccttgtgctaagagcttctggagcaagaccttcggaatagatcatttacagcagtgggtcactaccatagcaggagggcgtttccctagtgggcactgtgaaggcccttcagttcctgagctcagacatggctgacatccatccagagaacctggtttcattccacactggctattgtgctctgatgccagcctcctggtttgggcctggctaggtcttaggttgaccctaggaggaagcacggggccttatctcctccctcagcccctgcagagtattggggaaatagtacaggttccagatggagggacgctcctacatggccatcccctaggtgtctagggtgtgactagtaaggtcacctggttaggaaccacggttatcagttcttacaaagaggcccatccacactggcacagcattcatatgggggcttatttttaggtctcccaccttctacctgccaacacaaaatgctgaatgaaactggaacacacacacagaggcatgcacgcgcgcgcccgcacgagctgagggggatgtcatgagaggagttaagggcagccatggtttcctaaaagccacgcgggagtagtgatcacggacagcatgaaggaggcacggtcctcctgtttcagagatgcatgtggcacctggtgacacaagagcagtccagataccctgtgggttcaggggttcctgagggcttcctaggtatggggctttgtgctaggcattatccaaagcaaattcagctagcctagaagtacgcttggcaggctccgcgcgtggccatttctagctgcggagaagtcactcctctcaactgacagaactggcaataaagcgcctaaattctaaatacatgagtccctctctcatcctgtacctgcgaatggcatggcggcagcatctgtttgagagaatgtggcccactttaacccactgtgcctgtgggcaacaggtcccagctggggagggtgcccactcctctggaagtcgctgtctgttcattgtaaaactctcatttctctgcgcctgtggcctctgccagccagcggtggggagcctctggggagtgggagggaagaagggagagaagggggggggagagcactccttcctgccctccccacctccccgcggcctgggaaaaggcagcatattgaggcgcggggctctcagcatcaggccccgggatgctaatgagggcgagcgcgttcccacagcccggacattgtgccgcgcggcccacctgctcctcggggagcgaccattgtgcccgcgccaattcacaggcaatttagcgtgcgctaatgggccggcgcctttgtgcggccggcgccgccattggccgccgagtgtgggaacggccgcggcgcccggaccccaggcgccgggccgctgcccgcgcctatatagggctggcgtgctggggtccaggtcgcgccagtccgggacgcctggctctgtccgctccgctccgctccgctcgctaatcgcctccagagctccaggccttaagaggcaggcaggcttaattaagccaccatgaccacatttttcaccagcgtccctccctggattcaagatgcaaagcaggaggaggaagtgggctggaaactagttcccaggcctcggggccgggaggcagagagtcaagtgaagtgccaatgtgaaatctcggggacaccattttcaaatggggagaagctaaggcctcacagccttccccatccggagcagagaccatatagctgtcctcagctgcactgcggcaaggcttttgcctccaagtacaagctgtataggcacatggccacccactcggcccagaaaccccaccagtgcatgtactgtgacaagatgtttcaccgaaaggaccatctgcggaaccacttgcagacccatgaccccaacaaagaggccctccactgctctgagtgtggtaagaattataatacaaagctgggataccgtcgtcacctggccatgcatgctgccagcagtggtgatctcagctgcaaggtgtgcctgcagacctttgagagtacccaggccctattggagcacctgaaggctcactcacgccgggtagcaggaggtgctaaggagaagaagcacccctgtgaccattgtgacaggcggttctatactcggaaggatgtccgacggcacctagtggtgcacacaggtcgtaaggacttcctgtgtcagtactgtgcccagagatttggccgcaaggatcacctgacacgccatgtcaagaagagccactcacaggaactgctcaagatcaagacagagccagtggatatgttaggcttgctcagctgtagctctacagtcagtgtaaaggaagagctgagccctgtgctttgcatggcctctcgggacgtgatgggggctaaggcctttcctggcatgttgcccatgggtatgtatggtgcccacatccctaccatgcccagtgcgggcatgccacactccctggtgcacaacacactgcccatgggtatgagttaccctctggaatcttctcctatctcctcctcagctcagctccctccaaaataccagcttggatctacctcatacttgcccgacaaactgcccaaagtggaggtggatagttttctggcagagcttcctggaagcctgtctctctcctcggctgaacctcagcccgcctcacctcagccggcggcagctgcagccctcctggatgaagcactgctcgccaagagtcccgccaacctctccgaggccctctgcgctgctaatgtggacttttcccacttactgggctttcttccgctcaacctacccccatgtaacccaccaggggccacaggaggcttggttatgggctactcccaagctgaggcacagcctttgctcaccactttgcaggctcagcctcaagattccgctggagctgggggacccctgaactttgggcctctgcactccttacctcctgtcttcacctctggcctgagtaccaccaccctgcctcgtttccaccaagcattccagggaagcggagctactaacttcagcctgctgaagcaggctggagacgtggaggagaaccctggacctgtgagcaagggcgaggaggataacatggccatcatcaaggagttcatgcgcttcaaggtgcacatggagggctccgtgaacggccacgagttcgagatcgagggcgagggcgagggccgcccctacgagggcacccagaccgccaagctgaaggtgaccaagggtggccccctgcccttcgcctgggacatcctgtcccctcagttcatgtacggctccaaggcctacgtgaagcaccccgctgacatccccgactacttgaagctgtccttccccgagggcttcaagtgggagcgcgtgatgaacttcgaggacggcggcgtggtgaccgtgacccaggactcctccctgcaggacggcgagttcatctacaaggtgaagctgcgcggcaccaacttcccctccgacggccccgtaatgcagaagaagaccatgggctgggaggcctcctccgagcggatgtaccccgaggacggcgccctgaagggcgagatcaagcagaggctgaagctgaaggacggcggccactacgacgctgaggtcaagaccacctacaaggccaagaagcccgtgcagctgcccggcgcctacaacgtcaacatcaagttggacatcacctcccacaacgaggactacaccatcgtggaacagtacgaacgcgccgagggccgccactccaccggcggcatggacgagctgtacaaggatatccctccaaagaagaagagaaaggtgtaaggcgcgcctagggataacagggtaattgtttgaatgaggcttcagtactttacagaatcgttgcctgcacatcttggaaacacttgctgggattacttcgacttcttaacccaacagaaggctcgagaaggtatattgctgttgacagtgagcgcgctgtgtatattgtaacgttatagtgaagccacagatgtataacgttacaatatacacagcatgcctactgcctcggacttcaaggggctagaattcgagcaattatcttgtttactaaaactgaataccttgctatctctttgatacatttttacaaagctgaattaaaatggtataaattaaatcactctagtaataaaggatcctttatcttcattggatccgtgtgttggttttttgtgtgcggcccgtctagacc